European Patent Application EP 4 613 867 A2, published September 10, 2025. Title: NOVEL HIGH FIDELITY RNA-PROGRAMMABLE ENDONUCLEASE SYSTEMS AND USES THEREOF. Applicant: CRISPR THERAPEUTICS AG. Application EP. The sequence listing filed with the application follows.

SEQUENCE LISTING (133 sequences)

SEQ ID NO: 1 - protein, 1053 aa, synthetic construct
  REGION 406: note = X can be any of these amino acids: E, G,S,T,A, D
  REGION 412: note = X can be any of these amino acids: D,G,S,T,A,E
  REGION 416: note = X can be any of these amino acids: A, G, S, T, D, E
  REGION 420: note = X can be any of these amino acids: R, A, G, S, T, D, E
  source 1..1053: note = The sequence CANNOT be where X equals the following combination - 406: E, 412: D, 416: A, and 420: R; note = M-SauCas9_X; note = Synthetic
MKRNYILGLDIGITSVGYGIIDYETRDVIDAGVRLFKEANVENNEGRRSKRGARRLKRRRRHRIQRVKKLLFDYNLLTDHSELSGINPYEARVKGLSQKLSEEEFSAALLHLAKRRGVHNVNEVEEDTGNELSTKEQISRNSKALEEKYVAELQLERLKKDGEVRGSINRFKTSDYVKEAKQLLKVQKAYHQLDQSFIDTYIDLLETRRTYYEGPGEGSPFGWKDIKEWYEMLMGHCTYFPEELRSVKYAYNADLYNALNDLNNLVITRDENEKLEYYEKFQIIENVFKQKKKPTLKQIAKEILVNEEDIKGYRVTSTGKPEFTNLKVYHDIKDITARKEIIENAELLDQIAKILTIYQSSEDIQEELTNLNSELTQEEIEQISNLKGYTGTHNLSLKAINLILDXLWHTNXNQIXIFNXLKLVPKKVDLSQQKEIPTTLVDDFILSPVVKRSFIQSIKVINAIIKKYGLPNDIIIELAREKNSKDAQKMINEMQKRNRQTNERIEEIIRTTGKENAKYLIEKIKLHDMQEGKCLYSLEAIPLEDLLNNPFNYEVDHIIPRSVSFDNSFNNKVLVKQEENSKKGNRTPFQYLSSSDSKISYETFKKHILNLAKGKGRISKTKKEYLLEERDINRFSVQKDFINRNLVDTRYATRGLMNLLRSYFRVNNLDVKVKSINGGFTSFLRRKWKFKKERNKGYKHHAEDALIIANADFIFKEWKKLDKAKKVMENQMFEEKQAESMPEIETEQEYKEIFITPHQIKHIKDFKDYKYSHRVDKKPNRELINDTLYSTRKDDKGNTLIVNNLNGLYDKDNDKLKKLINKSPEKLLMYHHDPQTYQKLKLIMEQYGDEKNPLYKYYEETGNYLTKYSKKDNGPVIKKIKYYGNKLNAHLDITDDYPNSRNKVVKLSLKPYRFDVYLDNGVYKFVTVKNLDVIKKENYYEVNSKCYEEAKKLKKISNQAEFIASFYNNDLIKINGELYRVIGVNNDLLNRIEVNMIDITYREYLENMNDKRPPRIIKTIASKTQSIKKYSTDILGNLYEVKSKKHPQIIKKG

SEQ ID NO: 2 - protein, 1056 aa, synthetic construct
  REGION 239: note = X can be any of these amino acids: C, S, A
  REGION 401: note = X can be any of these amino acids: C, S, A
  REGION 408: note = X can be any of these amino acids: E, G,S,T,A,D
  REGION 414: note = X can be any of these amino acids: R, G,S,T,A, D, E
  REGION 418: note = X can be any of these amino acids: E, G, S, T, A, D
  REGION 422: note = X can be any of these amino acids: H, A, G, S, T, D, E
  source 1..1056: note = Synthetic; note = The sequence CANNOT be where X equals the following combination - 408: E, 414: R, 418: E, 422: H, 239: C, and 401: C; note = M-SluCas9_x
MNQKFILGLDIGITSVGYGLIDYETKNIIDAGVRLFPEANVENNEGRRSKRGSRRLKRRRIHRLERVKKLLEDYNLLDQSQIPQSTNPYAIRVKGLSEALSKDELVIALLHIAKRRGIHKIDVIDSNDDVGNELSTKEQLNKNSKLLKDKFVCQIQLERMNEGQVRGEKNRFKTADIIKEIIQLLNVQKNFHQLDENFINKYIELVEMRREYFEGPGKGSPYGWEGDPKAWYETLMGHXTYFPDELRSVKYAYSADLFNALNDLNNLVIQRDGLSKLEYHEKYHIIENVFKQKKKPTLKQIANEINVNPEDIKGYRITKSGKPQFTEFKLYHDLKSVLFDQSILENEDVLDQIAEILTIYQDKDSIKSKLTELDILLNEEDKENIAQLTGYTGTHRLSLKXIRLVLEXQWYSSXNQMXIFTXLNIKPKKINLTAANKIPKAMIDEFILSPVVKRTFGQAINLINKIIEKYGVPEDIIIELARENNSKDKQKFINEMQKKNENTRKRINEIIGKYGNQNAKRLVEKIRLHDEQEGKCLYSLESIPLEDLLNNPNHYEVDHIIPRSVSFDNSYHNKVLVKQSENSKKSNLTPYQYFNSGKSKLSYNQFKQHILNLSKSQDRISKKKKEYLLEERDINKFEVQKEFINRNLVDTRYATRELTNYLKAYFSANNMNVKVKTINGSFTDYLRKVWKFKKERNHGYKHHAEDALIIANADFLFKENKKLKAVNSVLEKPEIETKQLDIQVDSEDNYSEMFIIPKQVQDIKDFRNFKYSHRVDKKPNRQLINDTLYSTRKKDNSTYIVQTIKDIYAKDNTTLKKQFDKSPEKFLMYQHDPRTFEKLEVIMKQYANEKNPLAKYHEETGEYLTKYSKKNNGPIVKSLKYIGNKLGSHLDVTHQFKSSTKKLVKLSIKPYRFDVYLTDKGYKFITISYLDVLKKDNYYYIPEQKYDKLKLGKAIDKNAKFIASFYKNDLIKLDGEIYKIIGVNSDTRNMIELDLPDIRYKEYCELNNIKGEPRIKKTIGKKVNSIEKLTTDVLGNVFTNTQYTKPQLLFKRGNGG

SEQ ID NO: 3 - protein, 1054 aa, synthetic construct
  REGION 239: note = X can be any of these amino acids: C, S, A
  REGION 401: note = X can be any of these amino acids: C, S, A
  REGION 408: note = X can be any of these amino acids: E, G,S,T,A,D
  REGION 414: note = X can be any of these amino acids: R, G,S,T,A, D, E
  REGION 418: note = X can be any of these amino acids: E, G, S, T, A, D
  REGION 422: note = X can be any of these amino acids: Y, A, G, S, T, D, E
  source 1..1054: note = Synthetic; note = The sequence CANNOT be where X equals the following combination - 408:E, 414: R, 418: E, 422: Y, 239: C, and 401:C; note = M-SpaCas9_X
MKEKYILGLDLGITSVGYGIINFETKKIIDAGVRLFPEANVDNNEGRRSKRGSRRLKRRRIHRLERVKLLLTEYDLINKEQIPTSNNPYQIRVKGLSEILSKDELAIALLHLAKRRGIHNINVSSEDEDASNELSTKEQINRNNKLLKDKYVCEVQLQRLKEGQIRGEKNRFKTTDILKEIDQLLKVQKDYHNLDIDFINQYKEIVETRREYFEGPGQGSPFGWNGDLKKWYEMLMGHXTYFPQELRSVKYAYSADLFNALNDLNNLIIQRDNSEKLEYHEKYHIIENVFKQKKKPTLKQIAKEIGVNPEDIKGYRITKSGTPQFTEFKLYHDLKSIVFDKSILENEAILDQIAEILTIYQDEQSIKEELNKLPEILNEQDKAEIAKLIGYNGTHRLSLKXIHLINEXLWQTSXNQMXIFNXLNIKPNKVDLSEQNKIPKDMVNDFILSPVVKRTFIQSINVINKVIEKYGIPEDIIIELARENNSDDRKKFINNLQKKNEATRKRINEIIGQTGNQNAKRIVEKIRLHDQQEGKCLYSLESIALMDLLNNPQNYEVDHIIPRSVAFDNSIHNKVLVKQIENSKKGNRTPYQYLNSSDAKLSYNQFKQHILNLSKSKDRISKKKKDYLLEERDINKFEVQKEFINRNLVDTRYATRELTSYLKAYFSANNMDVKVKTINGSFTNHLRKVWRFDKYRNHGYKHHAEDALIIANADFLFKENKKLQNTNKILEKPTIENNTKKVTVEKEEDYNNVFETPKLVEDIKQYRDYKFSHRVDKKPNRQLINDTLYSTRMKDEHDYIVQTITDIYGKDNTNLKKQFNKNPEKFLMYQNDPKTFEKLSIIMKQYSDEKNPLAKYYEETGEYLTKYSKKNNGPIVKKIKLLGNKVGNHLDVTNKYENSTKKLVKLSIKNYRFDVYLTEKGYKFVTIAYLNVFKKDNYYYIPKDKYQELKEKKKIKDTDQFIASFYKNDLIKLNGDLYKIIGVNSDDRNIIELDYYDIKYKDYCEINNIKGEPRIKKTIGKKTESIEKFTTDVLGNLYLHSTEKAPQLIFKRGL

SEQ ID NO: 4 - protein, 1051 aa, synthetic construct
  REGION 239: note = X can be any of these amino acids: C, S, A
  REGION 401: note = X can be any of these amino acids: C, S, A
  REGION 408: note = X can be any of these amino acids: D, G,S,T,A,E
  REGION 414: note = X can be any of these amino acids: L, G,S,T,A, D, E
  REGION 418: note = X can be any of these amino acids: E, G, S, T, A, D
  REGION 422: note = X can be any of these amino acids: K, A, G, S, T, D, E
  source 1..1051: note = The sequence CANNOT be where X equals the following combination - 408: D, 414: L, 418: E, 422: K, 239: C, and 401: C; note = Synthetic; note = M-ShyCas9_X
MNNYILGLDIGITSVGYGIVDSDTREIKDAGVRLFPEANVDNNEGRRSKRGARRLKRRRIHRLDRVKHLLAEYDLLDLTNIPKSTNPYQTRVKGLNEKLSKDELVIALLHIAKRRGIHNVNVMMDDNDSGNELSTKDQLKKNAKALSDKYVCELQLERFEQDYKVRGEKNRFKTEDFVREARKLLETQSKFFEIDQTFIMRYIELIETRREYFEGPGKGSPFGWEGNIKKWFEQMMGHXTYFPEELRSVKYSYSAELFNALNDLNNLVITRDEDAKLNYGEKFQIIENVFKQKKTPNLKQIAIEIGVHETEIKGYRVNKSGKPEFTQFKLYHDLKNIFKDPKYLNDIQLMDNIAEIITIYQDAESIIKELNQLPELLSEREKEKISALSGYSGTHRLSLKXINLLLDXLWESSXNQMXLFTXLNLKPKKIDLSQQHKIPSKLVDDFILSPVVKRAFIQSIQVVNAIIDKYGLPEDIIIELARENNSDDRRKFLNQLQKQNEETRKQVEKVLREYGNDNAKRIVQKIKLHNMQEGKCLYSLKDIPLEDLLRNPHHYEVDHIIPRSVAFDNSMHNKVLVRADENSKKGNRTPYQYLNSSESSLSYNEFKQHILNLSKTKDRITKKKREYLLEERDINKFDVQKEFINRNLVDTRYATRELTSLLKAYFSANNLDVKVKTINGSFTNYLRKVWKFDKDRNKGYKHHAEDALIIANADFLFKHNKKLRNINKVLDAPSKEVDKKRVTVQSEDEYNQIFEDTQKAQAIKKFEIRKFSHRVDKKPNRQLINDTLYSTRNIDGIEYVVESIKDIYSVNNDKVKTKFKKDPHRLLMYRNDPQTFEKFEKVFKQYESEKNPFAKYYEETGEKIRKFSKTGQGPYINKIKYLRERLGRHCDVTNKYINSRNKIVQLKIYSYRFDIYQYGNNYKMITISYIDLEQKSNYYYISREKYEQKKKDKQIDDSYKFIGSFYKNDIINYNGEMYRVIGVNDSEKNKIQLDMIDISIKDYMELNNIKKTGVIYKTIGKSTTHIEKYTTDILGNLYKAAPPKKPQLIFK

SEQ ID NO: 5 - protein, 1052 aa, synthetic construct
  REGION 241: note = X can be any of these amino acids: C, S, A
  REGION 403: note = X can be any of these amino acids: C, S, A
  REGION 410: note = X can be any of these amino acids: E, G, S, T, A, D
  REGION 416: note = X can be any of these amino acids: M, G,S,T,A, D, E, L
  REGION 420: note = X can be any of these amino acids: E, G, S, T, A, D
  REGION 424: note = X can be any of these amino acids: Y, A, G, S, T, D, E
  source 1..1052: note = The sequence CANNOT be where X equals the following combination - 410: E, 416: M, 420: E, 424: Y, 241: C, and 403: C; note = Synthetic; note = M-SmiCas9_X
MEKDYILGLDIGIGSVGYGLIDYDTKSIIDAGVRLFPEANADNNLGRRAKRGARRLKRRRIHRLERVKSLLSEYKIISGLAPTNNQPYNIRVKGLTEQLTKDELAVALLHIAKRRGIHNVDVAADKEETASDSLSTKDQINKNAKFLESRYVCELQKERLENEGHVRGVENRFLTKDIVREAKKIIDTQMQYYPEIDETFKEKYISLVETRREYYEGPGKGSPYGWDADVKKWYQLMMGHXTYFPVEFRSVKYAYTADLYNALNDLNNLTIARDDNPKLEYHEKYHIIENVFKQKRNPTLKQIAKEIGVNDINISGYRVTKSGKPQFTSFKLFHDLKKVVKDHAILDDIDLLNQIAEILTIYQDKDSIVAELGQLEYLMSEADKQSISELTGYTGTHSLSLKXMNMIIDXLWHSSXNQMXVFTXLNMRPKKYELKGYQRIPTDMIDDAILSPVVKRSFKQAIGVVNAIIKKYGLPKDIIIELARESNSAEKSRYLRAIQKKNEKTRERIEAIIKEYGNENAKGLVQKIKLHDAQEGKCLYSLKDIPLEDLLRNPNNYDIDHIIPRSVSFDDSMHNKVLVRREQNAKKNNQTPYQYLTSGYADIKYSVFKQHVLNLAENKDRMTKKKREYLLEERNINKYDVQKEFINRNLVDTRYTTRELTTLLKTYFTINNLDVKVKTINGSFTDFLRKRWGFKKNRDEGYKHHAEDALIIANADYLFKEHKLLKEIKDVSDLAGDERNSNVKDEDQYEEVFGGYFKIEDIKKYKIKKFSHRVDKKPNRQLINDTIYSTRVKDDKRYLINTLKNLYDKSNGDLKERMQKDPESLLMYHHDPQTFEKLKIVMSQYENEKNPLAKYFEETGQYLTKYAKHDNGPAIHKIKYYGNKLVEHLDITKNYHNPQNKVVQLSQKSFRFDVYQTDKGYKFISIAYLTLKNEKNYYAISQEKYDQLKSEKKISNNAVFIGSFYTSDIIEINNEKFRVIGVNSDKNNLIEVDRIDIRQKEFIELEEEKKNNRIKVTIGRKTTNIEKFHTDILGNMYKSKRPKAPQLVFKKG

SEQ ID NO: 6 - protein, 1053 aa, synthetic construct
  source 1..1053: note = M-SauCas9R420A; note = Synthetic
MKRNYILGLDIGITSVGYGIIDYETRDVIDAGVRLFKEANVENNEGRRSKRGARRLKRRRRHRIQRVKKLLFDYNLLTDHSELSGINPYEARVKGLSQKLSEEEFSAALLHLAKRRGVHNVNEVEEDTGNELSTKEQISRNSKALEEKYVAELQLERLKKDGEVRGSINRFKTSDYVKEAKQLLKVQKAYHQLDQSFIDTYIDLLETRRTYYEGPGEGSPFGWKDIKEWYEMLMGHCTYFPEELRSVKYAYNADLYNALNDLNNLVITRDENEKLEYYEKFQIIENVFKQKKKPTLKQIAKEILVNEEDIKGYRVTSTGKPEFTNLKVYHDIKDITARKEIIENAELLDQIAKILTIYQSSEDIQEELTNLNSELTQEEIEQISNLKGYTGTHNLSLKAINLILDELWHTNDNQIAIFNALKLVPKKVDLSQQKEIPTTLVDDFILSPVVKRSFIQSIKVINAIIKKYGLPNDIIIELAREKNSKDAQKMINEMQKRNRQTNERIEEIIRTTGKENAKYLIEKIKLHDMQEGKCLYSLEAIPLEDLLNNPFNYEVDHIIPRSVSFDNSFNNKVLVKQEENSKKGNRTPFQYLSSSDSKISYETFKKHILNLAKGKGRISKTKKEYLLEERDINRFSVQKDFINRNLVDTRYATRGLMNLLRSYFRVNNLDVKVKSINGGFTSFLRRKWKFKKERNKGYKHHAEDALIIANADFIFKEWKKLDKAKKVMENQMFEEKQAESMPEIETEQEYKEIFITPHQIKHIKDFKDYKYSHRVDKKPNRELINDTLYSTRKDDKGNTLIVNNLNGLYDKDNDKLKKLINKSPEKLLMYHHDPQTYQKLKLIMEQYGDEKNPLYKYYEETGNYLTKYSKKDNGPVIKKIKYYGNKLNAHLDITDDYPNSRNKVVKLSLKPYRFDVYLDNGVYKFVTVKNLDVIKKENYYEVNSKCYEEAKKLKKISNQAEFIASFYNNDLIKINGELYRVIGVNNDLLNRIEVNMIDITYREYLENMNDKRPPRIIKTIASKTQSIKKYSTDILGNLYEVKSKKHPQIIKKG

SEQ ID NO: 7 - protein, 1056 aa, synthetic construct
  source 1..1056: note = M-SluCas9R414A; note = Synthetic
MNQKFILGLDIGITSVGYGLIDYETKNIIDAGVRLFPEANVENNEGRRSKRGSRRLKRRRIHRLERVKKLLEDYNLLDQSQIPQSTNPYAIRVKGLSEALSKDELVIALLHIAKRRGIHKIDVIDSNDDVGNELSTKEQLNKNSKLLKDKFVCQIQLERMNEGQVRGEKNRFKTADIIKEIIQLLNVQKNFHQLDENFINKYIELVEMRREYFEGPGKGSPYGWEGDPKAWYETLMGHCTYFPDELRSVKYAYSADLFNALNDLNNLVIQRDGLSKLEYHEKYHIIENVFKQKKKPTLKQIANEINVNPEDIKGYRITKSGKPQFTEFKLYHDLKSVLFDQSILENEDVLDQIAEILTIYQDKDSIKSKLTELDILLNEEDKENIAQLTGYTGTHRLSLKCIRLVLEEQWYSSANQMEIFTHLNIKPKKINLTAANKIPKAMIDEFILSPVVKRTFGQAINLINKIIEKYGVPEDIIIELARENNSKDKQKFINEMQKKNENTRKRINEIIGKYGNQNAKRLVEKIRLHDEQEGKCLYSLESIPLEDLLNNPNHYEVDHIIPRSVSFDNSYHNKVLVKQSENSKKSNLTPYQYFNSGKSKLSYNQFKQHILNLSKSQDRISKKKKEYLLEERDINKFEVQKEFINRNLVDTRYATRELTNYLKAYFSANNMNVKVKTINGSFTDYLRKVWKFKKERNHGYKHHAEDALIIANADFLFKENKKLKAVNSVLEKPEIETKQLDIQVDSEDNYSEMFIIPKQVQDIKDFRNFKYSHRVDKKPNRQLINDTLYSTRKKDNSTYIVQTIKDIYAKDNTTLKKQFDKSPEKFLMYQHDPRTFEKLEVIMKQYANEKNPLAKYHEETGEYLTKYSKKNNGPIVKSLKYIGNKLGSHLDVTHQFKSSTKKLVKLSIKPYRFDVYLTDKGYKFITISYLDVLKKDNYYYIPEQKYDKLKLGKAIDKNAKFIASFYKNDLIKLDGEIYKIIGVNSDTRNMIELDLPDIRYKEYCELNNIKGEPRIKKTIGKKVNSIEKLTTDVLGNVFTNTQYTKPQLLFKRGNGG

SEQ ID NO: 8 - protein, 1057 aa, synthetic construct
  source 1..1057: note = Synthetic; note = MGib11SpaCas9-3E410A
MNQKFILGLDIGITSVGYGLIDYETKNIIDAGVRLFPEANVENNEGRRSKRGSRRLKRRRIHRLERVKLLLTEYDLINKEQIPTSNNPYQIRVKGLSEILSKDELAIALLHLAKRRGIHNVDVAADKEETASDSLSTKDQINKNAKFLESRYVCELQKERLENEGHVRGVENRFLTKDIVREAKKIIDTQMQYYPEIDETFKEKYISLVETRREYFEGPGQGSPFGWNGDLKKWYEMLMGHCTYFPQELRSVKYAYSADLFNALNDLNNLIIQRDNSEKLEYHEKYHIIENVFKQKKKPTLKQIAKEIGVNPEDIKGYRITKSGTPEFTSFKLFHDLKKVVKDHAILDDIDLLNQIAEILTIYQDKDSIVAELGQLEYLMSEADKQSISELTGYTGTHSLSLKCMNMIIDALWHSSMNQMEVFTYLNMRPKKYELKGYQRIPTDMIDDAILSPVVKRTFIQSINVINKVIEKYGIPEDIIIELARENNSDDRKKFINNLQKKNEATRKRINEIIGQTGNQNAKRIVEKIRLHDQQEGKCLYSLESIPLEDLLNNPNHYEVDHIIPRSVSFDNSYHNKVLVKQSENSKKSNLTPYQYFNSGKSKLSYNQFKQHILNLSKSQDRISKKKKEYLLEERDINKFEVQKEFINRNLVDTRYATRELTSYLKAYFSANNMDVKVKTINGSFTNHLRKVWRFDKYRNHGYKHHAEDALIIANADFLFKENKKLQNTNKILEKPTIENNTKKVTVEKEEDYNNVFETPKLVEDIKQYRDYKFSHRVDKKPNRQLINDTLYSTRMKDEHDYIVQTITDIYGKDNTNLKKQFNKNPEKFLMYQNDPKTFEKLSIIMKQYSDEKNPLAKYYEETGEYLTKYSKKNNGPIVKKIKLLGNKVGNHLDVTNKYENSTKKLVKLSIKNYRFDVYLTEKGYKFVTIAYLNVFKKDNYYYIPKDKYQELKEKKKIKDTDQFIASFYKNDLIKLNGDLYKIIGVNSDDRNIIELDYYDIKYKDYCEINNIKGEPRIKKTIGKKTESIEKFTTDVLGNLYLHSTEKAPQLIFKRGL

SEQ ID NO: 9 - protein, 1056 aa, synthetic construct
  source 1..1056: note = Synthetic; note = SluCas9
MNQKFILGLDIGITSVGYGLIDYETKNIIDAGVRLFPEANVENNEGRRSKRGSRRLKRRRIHRLERVKKLLEDYNLLDQSQIPQSTNPYAIRVKGLSEALSKDELVIALLHIAKRRGIHKIDVIDSNDDVGNELSTKEQLNKNSKLLKDKFVCQIQLERMNEGQVRGEKNRFKTADIIKEIIQLLNVQKNFHQLDENFINKYIELVEMRREYFEGPGKGSPYGWEGDPKAWYETLMGHCTYFPDELRSVKYAYSADLFNALNDLNNLVIQRDGLSKLEYHEKYHIIENVFKQKKKPTLKQIANEINVNPEDIKGYRITKSGKPQFTEFKLYHDLKSVLFDQSILENEDVLDQIAEILTIYQDKDSIKSKLTELDILLNEEDKENIAQLTGYTGTHRLSLKCIRLVLEEQWYSSRNQMEIFTHLNIKPKKINLTAANKIPKAMIDEFILSPVVKRTFGQAINLINKIIEKYGVPEDIIIELARENNSKDKQKFINEMQKKNENTRKRINEIIGKYGNQNAKRLVEKIRLHDEQEGKCLYSLESIPLEDLLNNPNHYEVDHIIPRSVSFDNSYHNKVLVKQSENSKKSNLTPYQYFNSGKSKLSYNQFKQHILNLSKSQDRISKKKKEYLLEERDINKFEVQKEFINRNLVDTRYATRELTNYLKAYFSANNMNVKVKTINGSFTDYLRKVWKFKKERNHGYKHHAEDALIIANADFLFKENKKLKAVNSVLEKPEIETKQLDIQVDSEDNYSEMFIIPKQVQDIKDFRNFKYSHRVDKKPNRQLINDTLYSTRKKDNSTYIVQTIKDIYAKDNTTLKKQFDKSPEKFLMYQHDPRTFEKLEVIMKQYANEKNPLAKYHEETGEYLTKYSKKNNGPIVKSLKYIGNKLGSHLDVTHQFKSSTKKLVKLSIKPYRFDVYLTDKGYKFITISYLDVLKKDNYYYIPEQKYDKLKLGKAIDKNAKFIASFYKNDLIKLDGEIYKIIGVNSDTRNMIELDLPDIRYKEYCELNNIKGEPRIKKTIGKKVNSIEKLTTDVLGNVFTNTQYTKPQLLFKRGNGG

SEQ ID NO: 10 - RNA, 150 nt, synthetic construct
  source 1..150: mol_type = other RNA; note = sgRNA_Ex1; note = Synthetic
ggtgaacgtggatgaagttggttttagtactctggaaacagaatctactgaaacaagacaatatgtcgtgtttatcccatcaatttattggtgggatttttttctagcataaccccttggggcctctaaacgggtcttgaggggtttttt

SEQ ID NO: 11 - DNA, 28 bp, synthetic construct
  source 1..28: mol_type = other DNA; note = Synthetic; note = R01-1-A
ggtgaacgtggatgaagttgtggggtac

SEQ ID NO: 12 - DNA, 33 bp, synthetic construct
  source 1..33: mol_type = other DNA; note = Synthetic; note = R01-1-B
gcggtaccccacaacttcatccacgttcaccgg

SEQ ID NO: 13 - DNA, 28 bp, synthetic construct
  source 1..28: mol_type = other DNA; note = Synthetic; note = R01-2-A
agtgaacgtggatgaagttgtggggtac

SEQ ID NO: 14 - DNA, 33 bp, synthetic construct
  source 1..33: mol_type = other DNA; note = R01-2-B; note = Synthetic
gcggtaccccacaacttcatccacgttcactgg

SEQ ID NO: 15 - DNA, 28 bp, synthetic construct
  source 1..28: mol_type = other DNA; note = R01-3-A; note = Synthetic
cgtgaacgtggatgaagttgtggggtac

SEQ ID NO: 16 - DNA, 33 bp, synthetic construct
  source 1..33: mol_type = other DNA; note = R01-3-B; note = Synthetic
gcggtaccccacaacttcatccacgttcacggg

SEQ ID NO: 17 - DNA, 28 bp, synthetic construct
  source 1..28: mol_type = other DNA; note = R01-4-A; note = Synthetic
tgtgaacgtggatgaagttgtggggtac

SEQ ID NO: 18 - DNA, 33 bp, synthetic construct
  source 1..33: mol_type = other DNA; note = R01-4-B; note = Synthetic
gcggtaccccacaacttcatccacgttcacagg

SEQ ID NO: 19 - DNA, 28 bp, synthetic construct
  source 1..28: mol_type = other DNA; note = Synthetic; note = R01-5-A
gatgaacgtggatgaagttgtggggtac

SEQ ID NO: 20 - DNA, 33 bp, synthetic construct
  source 1..33: mol_type = other DNA; note = R01-5-B; note = Synthetic
gcggtaccccacaacttcatccacgttcatcgg

SEQ ID NO: 21 - DNA, 28 bp, synthetic construct
  source 1..28: mol_type = other DNA; note = R01-6-A; note = Synthetic
gctgaacgtggatgaagttgtggggtac

SEQ ID NO: 22 - DNA, 33 bp, synthetic construct
  source 1..33: mol_type = other DNA; note = R01-6-B; note = Synthetic
gcggtaccccacaacttcatccacgttcagcgg

SEQ ID NO: 23 - DNA, 28 bp, synthetic construct
  source 1..28: mol_type = other DNA; note = R01-7-A; note = Synthetic
gttgaacgtggatgaagttgtggggtac

SEQ ID NO: 24 - DNA, 33 bp, synthetic construct
  source 1..33: mol_type = other DNA; note = R01-7-B; note = Synthetic
gcggtaccccacaacttcatccacgttcaacgg

SEQ ID NO: 25 - DNA, 28 bp, synthetic construct
  source 1..28: mol_type = other DNA; note = R01-8-A; note = Synthetic
ggagaacgtggatgaagttgtggggtac

SEQ ID NO: 26 - DNA, 33 bp, synthetic construct
  source 1..33: mol_type = other DNA; note = R01-8-B; note = Synthetic
gcggtaccccacaacttcatccacgttctccgg

SEQ ID NO: 27 - DNA, 28 bp, synthetic construct
  source 1..28: mol_type = other DNA; note = R01-9-A; note = Synthetic
ggcgaacgtggatgaagttgtggggtac

SEQ ID NO: 28 - DNA, 33 bp, synthetic construct
  source 1..33: mol_type = other DNA; note = R01-9-B; note = Synthetic
gcggtaccccacaacttcatccacgttcgccgg

SEQ ID NO: 29 - DNA, 28 bp, synthetic construct
  source 1..28: mol_type = other DNA; note = R01-10-A; note = Synthetic
ggggaacgtggatgaagttgtggggtac

SEQ ID NO: 30 - DNA, 33 bp, synthetic construct
  source 1..33: mol_type = other DNA; note = R01-10-B; note = Synthetic
gcggtaccccacaacttcatccacgttccccgg

SEQ ID NO: 31 - DNA, 28 bp, synthetic construct
  source 1..28: mol_type = other DNA; note = R01-11-A; note = Synthetic
ggtaaacgtggatgaagttgtggggtac

SEQ ID NO: 32 - DNA, 33 bp, synthetic construct
  source 1..33: mol_type = other DNA; note = R01-11-B; note = Synthetic
gcggtaccccacaacttcatccacgtttaccgg

SEQ ID NO: 33 - DNA, 28 bp, synthetic construct
  source 1..28: mol_type = other DNA; note = R01-12-A; note = Synthetic
ggtcaacgtggatgaagttgtggggtac

SEQ ID NO: 34 - DNA, 33 bp, synthetic construct
  source 1..33: mol_type = other DNA; note = R01-12-B; note = Synthetic
gcggtaccccacaacttcatccacgttgaccgg

SEQ ID NO: 35 - DNA, 28 bp, synthetic construct
  source 1..28: mol_type = other DNA; note = R01-13-A; note = Synthetic
ggttaacgtggatgaagttgtggggtac

SEQ ID NO: 36 - DNA, 33 bp, synthetic construct
  source 1..33: mol_type = other DNA; note = R01-13-B; note = Synthetic
gcggtaccccacaacttcatccacgttaaccgg

SEQ ID NO: 37 - DNA, 28 bp, synthetic construct
  source 1..28: mol_type = other DNA; note = R01-14-A; note = Synthetic
ggtgcacgtggatgaagttgtggggtac

SEQ ID NO: 38 - DNA, 33 bp, synthetic construct
  source 1..33: mol_type = other DNA; note = R01-14-B; note = Synthetic
gcggtaccccacaacttcatccacgtgcaccgg

SEQ ID NO: 39 - DNA, 28 bp, synthetic construct
  source 1..28: mol_type = other DNA; note = R01-15-A; note = Synthetic
ggtgtacgtggatgaagttgtggggtac

SEQ ID NO: 40 - DNA, 33 bp, synthetic construct
  source 1..33: mol_type = other DNA; note = R01-15-B; note = Synthetic
gcggtaccccacaacttcatccacgtacaccgg

SEQ ID NO: 41 - DNA, 28 bp, synthetic construct
  source 1..28: mol_type = other DNA; note = R01-16-A; note = Synthetic
ggtggacgtggatgaagttgtggggtac

SEQ ID NO: 42 - DNA, 33 bp, synthetic construct
  source 1..33: mol_type = other DNA; note = R01-16-B; note = Synthetic
gcggtaccccacaacttcatccacgtccaccgg

SEQ ID NO: 43 - DNA, 28 bp, synthetic construct
  source 1..28: mol_type = other DNA; note = R01-17-A; note = Synthetic
ggtgaccgtggatgaagttgtggggtac

SEQ ID NO: 44 - DNA, 33 bp, synthetic construct
  source 1..33: mol_type = other DNA; note = R01-17-B; note = Synthetic
gcggtaccccacaacttcatccacggtcaccgg

SEQ ID NO: 45 - DNA, 28 bp, synthetic construct
  source 1..28: mol_type = other DNA; note = R01-18-A; note = Synthetic
ggtgatcgtggatgaagttgtggggtac

SEQ ID NO: 46 - DNA, 33 bp, synthetic construct
  source 1..33: mol_type = other DNA; note = R01-18-B; note = Synthetic
gcggtaccccacaacttcatccacgatcaccgg

SEQ ID NO: 47 - DNA, 28 bp, synthetic construct
  source 1..28: mol_type = other DNA; note = R01-19-A; note = Synthetic
ggtgagcgtggatgaagttgtggggtac

SEQ ID NO: 48 - DNA, 33 bp, synthetic construct
  source 1..33: mol_type = other DNA; note = R01-19-B; note = Synthetic
gcggtaccccacaacttcatccacgctcaccgg

SEQ ID NO: 49 - DNA, 28 bp, synthetic construct
  source 1..28: mol_type = other DNA; note = R01-20-A; note = Synthetic
ggtgaaagtggatgaagttgtggggtac

SEQ ID NO: 50 - DNA, 33 bp, synthetic construct
  source 1..33: mol_type = other DNA; note = R01-20-B; note = Synthetic
gcggtaccccacaacttcatccactttcaccgg

SEQ ID NO: 51 - DNA, 28 bp, synthetic construct
  source 1..28: mol_type = other DNA; note = R01-21-A; note = Synthetic
ggtgaatgtggatgaagttgtggggtac

SEQ ID NO: 52 - DNA, 33 bp, synthetic construct
  source 1..33: mol_type = other DNA; note = R01-21-B; note = Synthetic
gcggtaccccacaacttcatccacattcaccgg

SEQ ID NO: 53 - DNA, 28 bp, synthetic construct
  source 1..28: mol_type = other DNA; note = R01-22-A; note = Synthetic
ggtgaaggtggatgaagttgtggggtac

SEQ ID NO: 54 - DNA, 33 bp, synthetic construct
  source 1..33: mol_type = other DNA; note = R01-22-B; note = Synthetic
gcggtaccccacaacttcatccaccttcaccgg

SEQ ID NO: 55 - DNA, 28 bp, synthetic construct
  source 1..28: mol_type = other DNA; note = R01-23-A; note = Synthetic
ggtgaacatggatgaagttgtggggtac

SEQ ID NO: 56 - DNA, 33 bp, synthetic construct
  source 1..33: mol_type = other DNA; note = R01-23-B; note = Synthetic
gcggtaccccacaacttcatccatgttcaccgg

SEQ ID NO: 57 - DNA, 28 bp, synthetic construct
  source 1..28: mol_type = other DNA; note = R01-24-A; note = Synthetic
ggtgaacctggatgaagttgtggggtac

SEQ ID NO: 58 - DNA, 33 bp, synthetic construct
  source 1..33: mol_type = other DNA; note = R01-24-B; note = Synthetic
gcggtaccccacaacttcatccaggttcaccgg

SEQ ID NO: 59 - DNA, 28 bp, synthetic construct
  source 1..28: mol_type = other DNA; note = R01-25-A; note = Synthetic
ggtgaacttggatgaagttgtggggtac

SEQ ID NO: 60 - DNA, 33 bp, synthetic construct
  source 1..33: mol_type = other DNA; note = R01-25-B; note = Synthetic
gcggtaccccacaacttcatccaagttcaccgg

SEQ ID NO: 61 - DNA, 28 bp, synthetic construct
  source 1..28: mol_type = other DNA; note = R01-26-A; note = Synthetic
ggtgaacgaggatgaagttgtggggtac

SEQ ID NO: 62 - DNA, 33 bp, synthetic construct
  source 1..33: mol_type = other DNA; note = R01-26-B; note = Synthetic
gcggtaccccacaacttcatcctcgttcaccgg

SEQ ID NO: 63 - DNA, 28 bp, synthetic construct
  source 1..28: mol_type = other DNA; note = R01-27-A; note = Synthetic
ggtgaacgcggatgaagttgtggggtac

SEQ ID NO: 64 - DNA, 33 bp, synthetic construct
  source 1..33: mol_type = other DNA; note = R01-27-B; note = Synthetic
gcggtaccccacaacttcatccgcgttcaccgg

SEQ ID NO: 65 - DNA, 28 bp, synthetic construct
  source 1..28: mol_type = other DNA; note = R01-28-A; note = Synthetic
ggtgaacggggatgaagttgtggggtac

SEQ ID NO: 66 - DNA, 33 bp, synthetic construct
  source 1..33: mol_type = other DNA; note = R01-28-B; note = Synthetic
gcggtaccccacaacttcatccccgttcaccgg

SEQ ID NO: 67 - DNA, 28 bp, synthetic construct
  source 1..28: mol_type = other DNA; note = R01-29-A; note = Synthetic
ggtgaacgtagatgaagttgtggggtac

SEQ ID NO: 68 - DNA, 33 bp, synthetic construct
  source 1..33: mol_type = other DNA; note = R01-29-B; note = Synthetic
gcggtaccccacaacttcatctacgttcaccgg

SEQ ID NO: 69 - DNA, 28 bp, synthetic construct
  source 1..28: mol_type = other DNA; note = R01-30-A; note = Synthetic
ggtgaacgtcgatgaagttgtggggtac

SEQ ID NO: 70 - DNA, 33 bp, synthetic construct
  source 1..33: mol_type = other DNA; note = R01-30-B; note = Synthetic
gcggtaccccacaacttcatcgacgttcaccgg

SEQ ID NO: 71 - DNA, 28 bp, synthetic construct
  source 1..28: mol_type = other DNA; note = R01-31-A; note = Synthetic
ggtgaacgttgatgaagttgtggggtac

SEQ ID NO: 72 - DNA, 33 bp, synthetic construct
  source 1..33: mol_type = other DNA; note = R01-31-B; note = Synthetic
gcggtaccccacaacttcatcaacgttcaccgg

SEQ ID NO: 73 - DNA, 28 bp, synthetic construct
  source 1..28: mol_type = other DNA; note = R01-32-A; note = Synthetic
ggtgaacgtgaatgaagttgtggggtac

SEQ ID NO: 74 - DNA, 33 bp, synthetic construct
  source 1..33: mol_type = other DNA; note = R01-32-B; note = Synthetic
gcggtaccccacaacttcattcacgttcaccgg

SEQ ID NO: 75 - DNA, 28 bp, synthetic construct
  source 1..28: mol_type = other DNA; note = R01-33-A; note = Synthetic
ggtgaacgtgcatgaagttgtggggtac

SEQ ID NO: 76 - DNA, 33 bp, synthetic construct
  source 1..33: mol_type = other DNA; note = R01-33-B; note = Synthetic
gcggtaccccacaacttcatgcacgttcaccgg

SEQ ID NO: 77 - DNA, 28 bp, synthetic construct
  source 1..28: mol_type = other DNA; note = R01-34-A; note = Synthetic
ggtgaacgtgtatgaagttgtggggtac

SEQ ID NO: 78 - DNA, 33 bp, synthetic construct
  source 1..33: mol_type = other DNA; note = R01-34-B; note = Synthetic
gcggtaccccacaacttcatacacgttcaccgg

SEQ ID NO: 79 - DNA, 28 bp, synthetic construct
  source 1..28: mol_type = other DNA; note = R01-35-A; note = Synthetic
ggtgaacgtggctgaagttgtggggtac

SEQ ID NO: 80 - DNA, 33 bp, synthetic construct
  source 1..33: mol_type = other DNA; note = R01-35-B; note = Synthetic
gcggtaccccacaacttcagccacgttcaccgg

SEQ ID NO: 81 - DNA, 28 bp, synthetic construct
  source 1..28: mol_type = other DNA; note = R01-36-A; note = Synthetic
ggtgaacgtggttgaagttgtggggtac

SEQ ID NO: 82 - DNA, 33 bp, synthetic construct
  source 1..33: mol_type = other DNA; note = R01-36-B; note = Synthetic
gcggtaccccacaacttcaaccacgttcaccgg

SEQ ID NO: 83 - DNA, 28 bp, synthetic construct
  source 1..28: mol_type = other DNA; note = R01-37-A; note = Synthetic
ggtgaacgtgggtgaagttgtggggtac

SEQ ID NO: 84 - DNA, 33 bp, synthetic construct
  source 1..33: mol_type = other DNA; note = R01-37-B; note = Synthetic
gcggtaccccacaacttcacccacgttcaccgg

SEQ ID NO: 85 - DNA, 28 bp, synthetic construct
  source 1..28: mol_type = other DNA; note = R01-38-A; note = Synthetic
ggtgaacgtggaagaagttgtggggtac

SEQ ID NO: 86 - DNA, 33 bp, synthetic construct
  source 1..33: mol_type = other DNA; note = R01-38-B; note = Synthetic
gcggtaccccacaacttcttccacgttcaccgg

SEQ ID NO: 87 - DNA, 28 bp, synthetic construct
  source 1..28: mol_type = other DNA; note = R01-39-A; note = Synthetic
ggtgaacgtggacgaagttgtggggtac

SEQ ID NO: 88 - DNA, 33 bp, synthetic construct
  source 1..33: mol_type = other DNA; note = R01-39-B; note = Synthetic
gcggtaccccacaacttcgtccacgttcaccgg

SEQ ID NO: 89 - DNA, 28 bp, synthetic construct
  source 1..28: mol_type = other DNA; note = R01-40-A; note = Synthetic
ggtgaacgtggaggaagttgtggggtac

SEQ ID NO: 90 - DNA, 33 bp, synthetic construct
  source 1..33: mol_type = other DNA; note = R01-40-B; note = Synthetic
gcggtaccccacaacttcctccacgttcaccgg

SEQ ID NO: 91 - DNA, 28 bp, synthetic construct
  source 1..28: mol_type = other DNA; note = R01-41-A; note = Synthetic
ggtgaacgtggataaagttgtggggtac

SEQ ID NO: 92 - DNA, 33 bp, synthetic construct
  source 1..33: mol_type = other DNA; note = R01-41-B; note = Synthetic
gcggtaccccacaactttatccacgttcaccgg

SEQ ID NO: 93 - DNA, 28 bp, synthetic construct
  source 1..28: mol_type = other DNA; note = R01-42-A; note = Synthetic
ggtgaacgtggatcaagttgtggggtac

SEQ ID NO: 94 - DNA, 33 bp, synthetic construct
  source 1..33: mol_type = other DNA; note = R01-42-B; note = Synthetic
gcggtaccccacaacttgatccacgttcaccgg

SEQ ID NO: 95 - DNA, 28 bp, synthetic construct
  source 1..28: mol_type = other DNA; note = R01-43-A; note = Synthetic
ggtgaacgtggattaagttgtggggtac

SEQ ID NO: 96 - DNA, 33 bp, synthetic construct
  source 1..33: mol_type = other DNA; note = R01-43-B; note = Synthetic
gcggtaccccacaacttaatccacgttcaccgg

SEQ ID NO: 97 - DNA, 28 bp, synthetic construct
  source 1..28: mol_type = other DNA; note = R01-44-A; note = Synthetic
ggtgaacgtggatgcagttgtggggtac

SEQ ID NO: 98 - DNA, 33 bp, synthetic construct
  source 1..33: mol_type = other DNA; note = R01-44-B; note = Synthetic
gcggtaccccacaactgcatccacgttcaccgg

SEQ ID NO: 99 - DNA, 28 bp, synthetic construct
  source 1..28: mol_type = other DNA; note = R01-45-A; note = Synthetic
ggtgaacgtggatgtagttgtggggtac

SEQ ID NO: 100 - DNA, 33 bp, synthetic construct
  source 1..33: mol_type = other DNA; note = R01-45-B; note = Synthetic
gcggtaccccacaactacatccacgttcaccgg

SEQ ID NO: 101 - DNA, 28 bp, synthetic construct
  source 1..28: mol_type = other DNA; note = R01-46-A; note = Synthetic
ggtgaacgtggatggagttgtggggtac

SEQ ID NO: 102 - DNA, 33 bp, synthetic construct
  source 1..33: mol_type = other DNA; note = R01-46-B; note = Synthetic
gcggtaccccacaactccatccacgttcaccgg

SEQ ID NO: 103 - DNA, 28 bp, synthetic construct
  source 1..28: mol_type = other DNA; note = R01-47-A; note = Synthetic
ggtgaacgtggatgacgttgtggggtac

SEQ ID NO: 104 - DNA, 33 bp, synthetic construct
  source 1..33: mol_type = other DNA; note = R01-47-B; note = Synthetic
gcggtaccccacaacgtcatccacgttcaccgg

SEQ ID NO: 105 - DNA, 28 bp, synthetic construct
  source 1..28: mol_type = other DNA; note = R01-48-A; note = Synthetic
ggtgaacgtggatgatgttgtggggtac

SEQ ID NO: 106 - DNA, 33 bp, synthetic construct
  source 1..33: mol_type = other DNA; note = R01-48-B; note = Synthetic
gcggtaccccacaacatcatccacgttcaccgg

SEQ ID NO: 107 - DNA, 28 bp, synthetic construct
  source 1..28: mol_type = other DNA; note = R01-49-A; note = Synthetic
ggtgaacgtggatgaggttgtggggtac

SEQ ID NO: 108 - DNA, 33 bp, synthetic construct
  source 1..33: mol_type = other DNA; note = R01-49-B; note = Synthetic
gcggtaccccacaacctcatccacgttcaccgg

SEQ ID NO: 109 - DNA, 27 bp, synthetic construct
  source 1..27: mol_type = other DNA; note = R01-50-A; note = Synthetic
ggtgaacgtggatgaaattgtggggta

SEQ ID NO: 110 - DNA, 33 bp, synthetic construct
  source 1..33: mol_type = other DNA; note = R01-50-B; note = Synthetic
gcggtaccccacaatttcatccacgttcaccgg

SEQ ID NO: 111 - DNA, 28 bp, synthetic construct
  source 1..28: mol_type = other DNA; note = R01-51-A; note = Synthetic
ggtgaacgtggatgaacttgtggggtac

SEQ ID NO: 112 - DNA, 33 bp, synthetic construct
  source 1..33: mol_type = other DNA; note = R01-51-B; note = Synthetic
gcggtaccccacaagttcatccacgttcaccgg

SEQ ID NO: 113 - DNA, 28 bp, synthetic construct
  source 1..28: mol_type = other DNA; note = R01-52-A; note = Synthetic
ggtgaacgtggatgaatttgtggggtac

SEQ ID NO: 114 - DNA, 33 bp, synthetic construct
  source 1..33: mol_type = other DNA; note = R01-52-B; note = Synthetic
gcggtaccccacaaattcatccacgttcaccgg

SEQ ID NO: 115 - DNA, 28 bp, synthetic construct
  source 1..28: mol_type = other DNA; note = R01-53-A; note = Synthetic
ggtgaacgtggatgaagatgtggggtac

SEQ ID NO: 116 - DNA, 33 bp, synthetic construct
  source 1..33: mol_type = other DNA; note = R01-53-B; note = Synthetic
gcggtaccccacatcttcatccacgttcaccgg

SEQ ID NO: 117 - DNA, 28 bp, synthetic construct
  source 1..28: mol_type = other DNA; note = R01-54-A; note = Synthetic
ggtgaacgtggatgaagctgtggggtac

SEQ ID NO: 118 - DNA, 33 bp, synthetic construct
  source 1..33: mol_type = other DNA; note = R01-54-B; note = Synthetic
gcggtaccccacagcttcatccacgttcaccgg

SEQ ID NO: 119 - DNA, 28 bp, synthetic construct
  source 1..28: mol_type = other DNA; note = R01-55-A; note = Synthetic
ggtgaacgtggatgaaggtgtggggtac

SEQ ID NO: 120 - DNA, 33 bp, synthetic construct
  source 1..33: mol_type = other DNA; note = R01-55-B; note = Synthetic
gcggtaccccacaccttcatccacgttcaccgg

SEQ ID NO: 121 - DNA, 28 bp, synthetic construct
  source 1..28: mol_type = other DNA; note = R01-56-A; note = Synthetic
ggtgaacgtggatgaagtagtggggtac

SEQ ID NO: 122 - DNA, 33 bp, synthetic construct
  source 1..33: mol_type = other DNA; note = R01-56-B; note = Synthetic
gcggtaccccactacttcatccacgttcaccgg

SEQ ID NO: 123 - DNA, 28 bp, synthetic construct
  source 1..28: mol_type = other DNA; note = R01-57-A; note = Synthetic
ggtgaacgtggatgaagtcgtggggtac

SEQ ID NO: 124 - DNA, 33 bp, synthetic construct
  source 1..33: mol_type = other DNA; note = R01-57-B; note = Synthetic
gcggtaccccacgacttcatccacgttcaccgg

SEQ ID NO: 125 - DNA, 28 bp, synthetic construct
  source 1..28: mol_type = other DNA; note = R01-58-A; note = Synthetic
ggtgaacgtggatgaagtggtggggtac

SEQ ID NO: 126 - DNA, 33 bp, synthetic construct
  source 1..33: mol_type = other DNA; note = R01-58-B; note = Synthetic
gcggtaccccaccacttcatccacgttcaccgg

SEQ ID NO: 127 - DNA, 28 bp, synthetic construct
  source 1..28: mol_type = other DNA; note = R01-59-A; note = Synthetic
ggtgaacgtggatgaagttatggggtac

SEQ ID NO: 128 - DNA, 33 bp, synthetic construct
  source 1..33: mol_type = other DNA; note = R01-59-B; note = Synthetic
gcggtaccccataacttcatccacgttcaccgg

SEQ ID NO: 129 - DNA, 28 bp, synthetic construct
  source 1..28: mol_type = other DNA; note = R01-60-A; note = Synthetic
ggtgaacgtggatgaagttctggggtac

SEQ ID NO: 130 - DNA, 33 bp, synthetic construct
  source 1..33: mol_type = other DNA; note = R01-60-B; note = Synthetic
gcggtaccccagaacttcatccacgttcaccgg

SEQ ID NO: 131 - DNA, 28 bp, synthetic construct
  source 1..28: mol_type = other DNA; note = R01-61-A; note = Synthetic
ggtgaacgtggatgaagttttggggtac

SEQ ID NO: 132 - DNA, 33 bp, synthetic construct
  source 1..33: mol_type = other DNA; note = R01-61-B; note = Synthetic
gcggtaccccaaaacttcatccacgttcaccgg

SEQ ID NO: 133 - protein, 1057 aa, synthetic construct
  source 1..1057: note = Gib11SpaCas9-1-M417L; note = Synthetic
MNQKFILGLDIGITSVGYGLIDYETKNIIDAGVRLFPEANVENNEGRRSKRGSRRLKRRRIHRLERVKLLLTEYDLINKEQIPTSNNPYQIRVKGLSEILSKDELAIALLHLAKRRGIHNVDVAADKEETASDSLSTKDQINKNAKFLESRYVCELQKERLENEGHVRGVENRFLTKDIVREAKKIIDTQMQYYPEIDETFKEKYISLVETRREYFEGPGQGSPFGWNGDLKKWYEMLMGHCTYFPQELRSVKYAYSADLFNALNDLNNLIIQRDNSEKLEYHEKYHIIENVFKQKKKPTLKQIAKEIGVNPEDIKGYRITKSGTPEFTSFKLFHDLKKVVKDHAILDDIDLLNQIAEILTIYQDKDSIVAELGQLEYLMSEADKQSISELTGYTGTHSLSLKCMNMIIDELWHSSLNQMEVFTYLNMRPKKYELKGYQRIPTDMIDDAILSPVVKRTFIQSINVINKVIEKYGIPEDIIIELARENNSDDRKKFINNLQKKNEATRKRINEIIGQTGNQNAKRIVEKIRLHDQQEGKCLYSLESIPLEDLLNNPNHYEVDHIIPRSVSFDNSYHNKVLVKQSENSKKSNLTPYQYFNSGKSKLSYNQFKQHILNLSKSQDRISKKKKEYLLEERDINKFEVQKEFINRNLVDTRYATRELTNYLKAYFSANNMNVKVKTINGSFTDYLRKVWKFKKERNHGYKHHAEDALIIANADFLFKENKKLKAVNSVLEKPEIETKQLDIQVDSEDNYSEMFIIPKQVQDIKDFRNFKYSHRVDKKPNRQLINDTLYSTRKKDNSTYIVQTIKDIYAKDNTTLKKQFDKSPEKFLMYQHDPRTFEKLEVIMKQYANEKNPLAKYHEETGEYLTKYSKKNNGPIVKSLKYIGNKLGSHLDVTHQFKSSTKKLVKLSIKNYRFDVYLTEKGYKFVTIAYLNVFKKDNYYYIPKDKYQELKEKKKIKDTDQFIASFYKNDLIKLNGDLYKIIGVNSDDRNIIELDYYDIKYKDYCEINNIKGEPRIKKTIGKKTESIEKFTTDVLGNLYLHSTEKAPQLIFKRGL